European Patent Specification EP 3 358 943 B1, published January 3, 2024. Title: Watermelon plants with Cucumber Vein Yellowing Virus (CVYV) resistance. Applicant: Nunhems B.V. The sequence listing filed with the application follows.

SEQUENCE LISTING (4 sequences)

SEQ ID NO: 1 - DNA, 151 bp, Citrullus lanatus
  SNP01 (76)..(76)
ggggcgaataaaataaaataaataaatttggtagggttggagtggaataaaggagattttattttatttggttgaagaaacaaaaagggaaaaattggaattaagggtttaaggagggagaggaattagggtttagtttaatcccaccctc

SEQ ID NO: 2 - DNA, 151 bp, Citrullus lanatus
  SNP02 (76)..(76)
tcagtcatagtatagtggaatatttgactgcaggtataagactcaacttcagaaagatccagaccttttttttaagagagagagagagagagagagagagagaactagaaacaacaatttccaccaaaagaatgaaaagagactaagactc

SEQ ID NO: 3 - DNA, 151 bp, Citrullus lanatus
  SNP03 (76)..(76)
cgagttggctattagagttgatcgttggagatgattgactgagttagttgctagaggtggtcgttgagttggttgccgaaggtattcgtcagggctagttgcgaagttgggctttggagaagtggagatagtcattgtagttgattgatgg

SEQ ID NO: 4 - DNA, 340 bp, Citrullus lanatus
  SNP04 (70)..(70)
tgaagttctacctccaaaactcctcaacagtagagaaggtatagatcggtcggatagacgcaccccagggggcttgcttagacttggcggatgggttatcgaaccaaaaggtccaagagtgctcaagagggtgaggctgatgcactatcgccgccgacaaattggacgagtcaaggtcgtcgtctccgacgatctctccttcctcaagttcctcatcttcatcaccgcctcgtcctctagggttttgatttgcaatggtattagaaagatcttccgtggatgtagctttgatcgtctcttcgactaccattttcctttcactacttgtggaattgagcgt